European Patent Application EP 4 397 685 A1, published July 10, 2024. Title: Anti-CD3 humanized antibody. Applicant: NOVOPROTEIN SCIENTIFIC INC. NOVOPROTEIN SCIENTIFIC (SHANGHAI) INC. The sequence listing filed with the application follows.

SEQUENCE LISTING (38 sequences)

SEQ ID NO: 1 - protein, 8 aa, Artificial Sequence
  huVH-CDR1
GFTFNKYA

SEQ ID NO: 2 - protein, 10 aa, Artificial Sequence
  huVH-CDR2
IRSKYNNYAT

SEQ ID NO: 3 - protein, 14 aa, Artificial Sequence
  huVH4-CDR3
HGNFGNSYISYWEY

SEQ ID NO: 4 - protein, 9 aa, Artificial Sequence
  huVL-CDR1
TGAVTSGNY

SEQ ID NO: 5 - protein, 3 aa, Artificial Sequence
  huVL-CDR2
GTK

SEQ ID NO: 6 - protein, 8 aa, Artificial Sequence
  HuVL4-CDR
VLWNSNRW

SEQ ID NO: 7 - protein, 125 aa, Artificial Sequence
  huVH4
EVQLVESGGGLVQPGGSLKLSCAASGFTFNKYAMNWVRQAPGKGLEWVARIRSKYNNYATYYADSVKDRFTISRDDSKNTAYLQMNNLKTEDTAVYYCVRHGNFGNSYISYWEYWGQGTLVTVSS

SEQ ID NO: 8 - protein, 109 aa, Artificial Sequence
  huVL4
QTVVTQEPSLTVSPGGTVTLTCGSSTGAVTSGNYPNWVQQKPGQAPRGLIGGTKFLAPGTPARFSGSLLGDKAALTLSGVQPEDEAEYYCVLWNSNRWVFGGGTKLTVL

SEQ ID NO: 9 - protein, 249 aa, Artificial Sequence
  Humanized CD3 single chain antibody huVH4VL4
EVQLVESGGGLVQPGGSLKLSCAASGFTFNKYAMNWVRQAPGKGLEWVARIRSKYNNYATYYADSVKDRFTISRDDSKNTAYLQMNNLKTEDTAVYYCVRHGNFGNSYISYWEYWGQGTLVTVSSGGGGSGGGGSGGGGSQTVVTQEPSLTVSPGGTVTLTCGSSTGAVTSGNYPNWVQQKPGQAPRGLIGGTKFLAPGTPARFSGSLLGDKAALTLSGVQPEDEAEYYCVLWNSNRWVFGGGTKLTVL

SEQ ID NO: 10 - protein, 14 aa, Artificial Sequence
  huVH3-CDR3
HGNFGNSYISYWRY

SEQ ID NO: 11 - protein, 8 aa, Artificial Sequence
  HuVL3-CDR3
VLWYSGRW

SEQ ID NO: 12 - protein, 125 aa, Artificial Sequence
  huVH3
EVQLVESGGGLVQPGGSLKLSCAASGFTFNKYAMNWVRQAPGKGLEWVARIRSKYNNYATYYADSVKDRFTISRDDSKNTAYLQMNNLKTEDTAVYYCVRHGNFGNSYISYWRYWGQGTLVTVSS

SEQ ID NO: 13 - protein, 109 aa, Artificial Sequence
  huVL3
QTVVTQEPSLTVSPGGTVTLTCGSSTGAVTSGNYPNWVQQKPGQAPRGLIGGTKFLAPGTPARFSGSLLGGKAALTLSGVQPEDEAEYYCVLWYSGRWVFGGGTKLTVL

SEQ ID NO: 14 - protein, 249 aa, Artificial Sequence
  Humanized CD3 single chain antibody huVH3VL3
EVQLVESGGGLVQPGGSLKLSCAASGFTFNKYAMNWVRQAPGKGLEWVARIRSKYNNYATYYADSVKDRFTISRDDSKNTAYLQMNNLKTEDTAVYYCVRHGNFGNSYISYWRYWGQGTLVTVSSGGGGSGGGGSGGGGSQTVVTQEPSLTVSPGGTVTLTCGSSTGAVTSGNYPNWVQQKPGQAPRGLIGGTKFLAPGTPARFSGSLLGGKAALTLSGVQPEDEAEYYCVLWYSGRWVFGGGTKLTVL

SEQ ID NO: 15 - protein, 14 aa, Artificial Sequence
  huVH2-CDR3
HGNFGNSYISYWQY

SEQ ID NO: 16 - protein, 8 aa, Artificial Sequence
  HuVL2-CDR3
VLWRSNRW

SEQ ID NO: 17 - protein, 125 aa, Artificial Sequence
  huVH2
EVQLVESGGGLVQPGGSLKLSCAASGFTFNKYAMNWVRQAPGKGLEWVARIRSKYNNYATYYADSVKDRFTISRDDSKNTAYLQMNNLKTEDTAVYYCVRHGNFGNSYISYWQYWGQGTLVTVSS

SEQ ID NO: 18 - protein, 109 aa, Artificial Sequence
  huVL2
QTVVTQEPSLTVSPGGTVTLTCGSSTGAVTSGNYPNWVQQKPGQAPRGLIGGTKFLAPGTPARFSGSLLGGKAALTLSGVQPEDEAEYYCVLWRSNRWVFGGGTKLTVL

SEQ ID NO: 19 - protein, 249 aa, Artificial Sequence
  Humanized CD3 single chain antibody huVH2VL2
EVQLVESGGGLVQPGGSLKLSCAASGFTFNKYAMNWVRQAPGKGLEWVARIRSKYNNYATYYADSVKDRFTISRDDSKNTAYLQMNNLKTEDTAVYYCVRHGNFGNSYISYWQYWGQGTLVTVSSGGGGSGGGGSGGGGSQTVVTQEPSLTVSPGGTVTLTCGSSTGAVTSGNYPNWVQQKPGQAPRGLIGGTKFLAPGTPARFSGSLLGGKAALTLSGVQPEDEAEYYCVLWRSNRWVFGGGTKLTVL

SEQ ID NO: 20 - protein, 14 aa, Artificial Sequence
  huVH1-CDR3
HGNFGNTYISYWAY

SEQ ID NO: 21 - protein, 8 aa, Artificial Sequence
  HuVL1-CDR3
VLWYSKRW

SEQ ID NO: 22 - protein, 125 aa, Artificial Sequence
  huVH1
EVQLVESGGGLVQPGGSLKLSCAASGFTFNKYAMNWVRQAPGKGLEWVARIRSKYNNYATYYADSVKDRFTISRDDSKNTAYLQMNNLKTEDTAVYYCVRHGNFGNTYISYWAYWGQGTLVTVSS

SEQ ID NO: 23 - protein, 109 aa, Artificial Sequence
  huVL1
QTVVTQEPSLTVSPGGTVTLTCGSSTGAVTSGNYPNWVQQKPGQAPRGLIGGTKFLAPGTPARFSGSLLGGKAALTLSGVQPEDEAEYYCVLWYSKRWVFGGGTKLTVL

SEQ ID NO: 24 - protein, 249 aa, Artificial Sequence
  Humanized CD3 single chain antibody huVH1VL1
EVQLVESGGGLVQPGGSLKLSCAASGFTFNKYAMNWVRQAPGKGLEWVARIRSKYNNYATYYADSVKDRFTISRDDSKNTAYLQMNNLKTEDTAVYYCVRHGNFGNTYISYWAYWGQGTLVTVSSGGGGSGGGGSGGGGSQTVVTQEPSLTVSPGGTVTLTCGSSTGAVTSGNYPNWVQQKPGQAPRGLIGGTKFLAPGTPARFSGSLLGGKAALTLSGVQPEDEAEYYCVLWYSKRWVFGGGTKLTVL

SEQ ID NO: 25 - protein, 330 aa, Artificial Sequence [sequence omitted]

SEQ ID NO: 26 - protein, 107 aa, Artificial Sequence
  Kappa Chain Constant region amino acid sequence
LTVAAPSVFIFPPSDEQLKSGTASVVCLLNNFYPREAKVQWKVDNALQSGNSQESVTEQDSKDSTYSLSSTLTLSKADYEKHKVYACEVTHQGLSSPVTKSFNRGEC

SEQ ID NO: 27 - protein, 450 aa, Artificial Sequence
  Heavy chain of OKT3 antibody
QVQLQQSGAELARPGASVKMSCKASGYTFTRYTMHWVKQRPGQGLEWIGYINPSRGYTNYNQKFKDKATLTTDKSSSTAYMQLSSLTSEDSAVYYCARYYDDHYCLDYWGQGTTLTVSSAKTTAPSVYPLAPVCGGTTGSSVTLGCLVKGYFPEPVTLTWNSGSLSSGVHTFPAVLQSDLYTLSSSVTVTSSTWPSQSITCNVAHPASSTKVDKKIEPRPKSCDKTHTCPPCPAPELLGGPSVFLFPPKPKDTLMISRTPEVTCVVVDVSHEDPEVKFNWYVDGVEVHNAKTKPREEQYNSTYRVVSVLTVLHQDWLNGKEYKCKVSNKALPAPIEKTISKAKGQPREPQVYTLPPSREEMTKNQVSLTCLVKGFYPSDIAVEWESNGQPENNYKTTPPVLDSDGSFFLYSKLTVDKSRWQQGNVFSCSVMHEALHNHYTQKSLSLSPGK

SEQ ID NO: 28 - protein, 213 aa, Artificial Sequence
  Light chain of OKT3 antibody
QIVLTQSPAIMSASPGEKVTMTCSASSSVSYMNWYQQKSGTSPKRWIYDTSKLASGVPAHFRGSGSGTSYSLTISGMEAEDAATYYCQQWSSNPFTFGSGTKLEINRADTAPTVSIFPPSSEQLTSGGASVVCFLNNFYPKDINVKWKIDGSERQNGVLNSWTDQDSKDSTYSMSSTLTLTKDEYERHNSYTCEATHKTSTSPIVKSFNRNEC

SEQ ID NO: 29 - protein, 14 aa, Artificial Sequence
  huVH5-CDR3
HGNLQNSYISYWAY

SEQ ID NO: 30 - protein, 9 aa, Artificial Sequence
  huVL5-CDR1
TGPVTGGNY

SEQ ID NO: 31 - protein, 8 aa, Artificial Sequence
  HuVL5-CDR3
VLWESNRW

SEQ ID NO: 32 - protein, 125 aa, Artificial Sequence
  huVH5
EVQLVESGGGLVQPGGSLKLSCAASGFTFNKYAMNWVRQAPGKGLEWVARIRSKYNNYATYYADSVKDRFTISRDDSKNTAYLQMNNLKTEDTAVYYCVRHGNLQNSYISYWAYWGQGTLVTVSS

SEQ ID NO: 33 - protein, 109 aa, Artificial Sequence.
  huVL5
QTVVTQEPSLTVSPGGTVTLTCGSSTGPVTGGNYPNWVQQKPGQAPRGLIGGTKFLAPGTPARFSGSLLGGKAALTLSGVQPEDEAEYYCVLWESNRWVFGGGTKLTVL

SEQ ID NO: 34 - protein, 215 aa, Artificial Sequence
  Humanized CD3 single chain antibody huVH5VL5
QTVVTQEPSLTVSPGGTVTLTCGSSTGPVTGGNYPNWVQQKPGQAPRGLIGGTKFLAPGTPARFSGSLLGGKAALTLSGVQPEDEAEYYCVLWESNRWVFGGGTKLTVLTVAAPSVFIFPPSDEQLKSGTASVVCLLNNFYPREAKVQWKVDNALQSGNSQESVTEQDSKDSTYSLSSTLTLSKADYEKHKVYACEVTHQGLSSPVTKSFNRGEC

SEQ ID NO: 35 - protein, 455 aa, Artificial Sequence
  Heavy chain of CD3 full-length antibody CQ54
EVQLVESGGGLVQPGGSLKLSCAASGFTFNKYAMNWVRQAPGKGLEWVARIRSKYNNYATYYADSVKDRFTISRDDSKNTAYLQMNNLKTEDTAVYYCVRHGNLQNSYISYWAYWGQGTLVTVSSASTKGPSVFPLAPSSKSTSGGTAALGCLVKDYFPEPVTVSWNSGALTSGVHTFPAVLQSSGLYSLSSVVTVPSSSLGTQTYICNVNHKPSNTKVDKKVEPKSCDKTHTCPPCPAPELLGGPSVFLFPPKPKDTLMISRTPEVTCVVVDVSHEDPEVKFNWYVDGVEVHNAKTKPREEQYNSTYRVVSVLTVLHQDWLNGKEYKCKVSNKALPAPIEKTISKAKGQPREPQVYTLPPSRDELTKNQVSLTCLVKGFYPSDIAVEWESNGQPENNYKTTPPVLDSDGSFFLYSKLTVDKSRWQQGNVFSCSVMHEALHNHYTQKSLSLSPGK

SEQ ID NO: 36 - protein, 215 aa, Artificial Sequence; identical to SEQ ID NO: 34
  Light chain of CD3 full-length antibody CQ54

SEQ ID NO: 37 - protein, 504 aa, Artificial Sequence
  Bispecific antibody SC30A of CD3 and CD19
DIQLTQSPASLAVSLGQRATISCKASQSVDYDGDSYLNWYQQIPGQPPKLLIYDASNLVSGIPPRFSGSGSGTDFTLNIHPVEKVDAATYHCQQSTEDPWTFGGGTKLEIKGGGGSGGGGSGGGGSQVQLQQSGAELVRPGSSVKISCKASGYAFSSYWMNWVKQRPGQGLEWIGQIWPGDGDTNYNGKFKGKATLTADESSSTAYMQLSSLASEDSAVYFCARRETTTVGRYYYAMDYWGQGTTVTVSSGGGGSEVQLVESGGGLVQPGGSLKLSCAASGFTFNKYAMNWVRQAPGKGLEWVARIRSKYNNYATYYADSVKDRFTISRDDSKNTAYLQMNNLKTEDTAVYYCVRHGNLQNSYISYWAYWGQGTLVTVSSGGGGSGGGGSGGGGSQTVVTQEPSLTVSPGGTVTLTCGSSTGPVTGGNYPNWVQQKPGQAPRGLIGGTKFLAPGTPARFSGSLLGGKAALTLSGVQPEDEAEYYCVLWESNRWVFGGGTKLTVL

SEQ ID NO: 38 - protein, 498 aa, Artificial Sequence
  BLMOA
DIQLTQSPASLAVSLGQRATISCKASQSVDYDGDSYLNWYQQIPGQPPKLLIYDASNLVSGIPPRFSGSGSGTDFTLNIHPVEKVDAATYHCQQSTEDPWTFGGGTKLEIKGGGGSGGGGSGGGGSQVQLQQSGAELVRPGSSVKISCKASGYAFSSYWMNWVKQRPGQGLEWIGQIWPGDGDTNYNGKFKGKATLTADESSSTAYMQLSSLASEDSAVYFCARRETTTVGRYYYAMDYWGQGTTVTVSSGGGGSDIKLQQSGAELARPGASVKMSCKTSGYTFTRYTMHWVKQRPGQGLEWIGYINPSRGYTNYNQKFKDKATLTTDKSSSTAYMQLSSLTSEDSAVYYCARYYDDHYCLDYWGQGTTLTVSSVEGGSGGSGGSGGSGGVDDIQLTQSPAIMSASPGEKVTMTCRASSSVSYMNWYQQKSGTSPKRWIYDTSKVASGVPYRFSGSGSGTSYSLTISSMEAEDAATYYCQQWSSNPLTFGAGTKLELK